European Patent Application EP 4 321 158 A1, published February 14, 2024. Title: Composition for Preventing or Treating Viral Infections Comprising Rottlerin as an active ingredient. Applicant: QVet. The sequence listing filed with the application follows.

SEQUENCE LISTING (8 sequences)

SEQ ID NO: 1 - DNA, 20 bp, Artificial Sequence
  SARS-CoV2-nsp10-F
ttgtgatcaactccgcgaac

SEQ ID NO: 2 - DNA, 20 bp, Artificial Sequence
  SARS-CoV2-nsp10-R
taagacgggctgcacttaca

SEQ ID NO: 3 - DNA, 25 bp, Artificial Sequence
  SARS-CoV2-nsp10-P
ccatgcttcagtcagctgatgcaca

SEQ ID NO: 4 - DNA, 21 bp, Artificial Sequence
  FCoV-F
acggtgtcttctgggttgcaa

SEQ ID NO: 5 - DNA, 23 bp, Artificial Sequence
  FCoV-R
ggctatgattgtatcctcaacat

SEQ ID NO: 6 - DNA, 20 bp, Artificial Sequence
  forward primer of PCV2 ORF3
ccttttttggcccgcagtat

SEQ ID NO: 7 - DNA, 20 bp, Artificial Sequence
  reverse primer of PCV2 ORF3
cagctgggacagcagttgag

SEQ ID NO: 8 - DNA, 25 bp, Artificial Sequence
  probe of PCV2 ORF3
ttaccagcaatcagaccccgttgga